European Patent Specification EP 3 765 525 B1, published July 19, 2023. Title: Anti-HER2 Biparatopic Antibody-Drug Conjugates and Methods of Use. Applicant: ZYMEWORKS INC. The sequence listing filed with the application follows.

SEQUENCE LISTING (89 sequences)

SEQ ID NO: 1 - protein, 217 aa, Artificial Sequence
  Artificial sequence
APELLGGPSVFLFPPKPKDTLMISRTPEVTCVVVDVSHEDPEVKFNWYVDGVEVHNAKTKPREEQYNSTYRVVSVLTVLHQDWLNGKEYKCKVSNKALPAPIEKTISKAKGQPREPQVYTLPPSRDELTKNQVSLTCLVKGFYPSDIAVEWESNGQPENNYKTTPPVLDSDGSFFLYSKLTVDKSRWQQGNVFSCSVMHEALHNHYTQKSLSLSPGK

SEQ ID NO: 2 - protein, 607 aa, Homo sapiens
TQVCTGTDMKLRLPASPETHLDMLRHLYQGCQVVQGNLELTYLPTNASLSFLQDIQEVQGYVLIAHNQVRQVPLQRLRIVRGTQLFEDNYALAVLDNGDPLNNTTPVTGASPGGLRELQLRSLTEILKGGVLIQRNPQLCYQDTILWKDIFHKNNQLALTLIDTNRSRACHPCSPMCKGSRCWGESSEDCQSLTRTVCAGGCARCKGPLPTDCCHEQCAAGCTGPKHSDCLACLHFNHSGICELHCPALVTYNTDTFESMPNPEGRYTFGASCVTACPYNYLSTDVGSCTLVCPLHNQEVTAEDGTQRCEKCSKPCARVCYGLGMEHLREVRAVTSANIQEFAGCKKIFGSLAFLPESFDGDPASNTAPLQPEQLQVFETLEEITGYLYISAWPDSLPDLSVFQNLQVIRGRILHNGAYSLTLQGLGISWLGLRSLRELGSGLALIHHNTHLCFVHTVPWDQLFRNPHQALLHTANRPEDECVGEGLACHQLCARGHCWGPGPTQCVNCSQFLRGQECVEECRVLQGLPREYVNARHCLPCHPECQPQNGSVTCFGPEADQCVACAHYKDPPFCVARCPSGVKPDLSYMPIWKFPDEEGACQPCPIN

SEQ ID NO: 3 - protein, 448 aa, Artificial Sequence
  Artificial sequence
EVQLVESGGGLVQPGGSLRLSCAASGFTFTDYTMDWVRQAPGKGLEWVADVNPNSGGSIYNQRFKGRFTLSVDRSKNTLYLQMNSLRAEDTAVYYCARNLGPSFYFDYWGQGTLVTVSSASTKGPSVFPLAPSSKSTSGGTAALGCLVKGYFPEPVTVSWNSGALTSGVHTFPAVLKSSGLYSLSSVVTVPSSSLGTQTYICNVNHKPSNTKVDKKVEPKSCDKTHTCPPCPAPELLGGPSVFLFPPKPKDTLMISRTPEVTCVVVDVSHEDPEVKFNWYVDGVEVHNAKTKPREEQYNSTYRVVSVLTVLHQDWLNGKEYKCKVSNKALPAPIEKTISKAKGQPREPQVYVLPPSRDELTKNQVSLLCLVKGFYPSDIAVEWESNGQPENNYLTWPPVLDSDGSFFLYSKLTVDKSRWQQGNVFSCSVMHEALHNHYTQKSLSLSPG

SEQ ID NO: 4 - DNA, 1344 bp, Artificial Sequence
  Artificial Sequence
gaagtgcagctggtcgaatctggaggaggactggtgcagccaggagggtccctgcgcctgtcttgcgccgctagtggcttcacttttaccgactacaccatggattgggtgcgacaggcacctggaaagggcctggagtgggtcgccgatgtgaacccaaatagcggaggctccatctacaaccagcggttcaagggccggttcaccctgtcagtggaccggagcaaaaacaccctgtatctgcagatgaatagcctgcgagccgaagatactgctgtgtactattgcgcccggaatctggggccctccttctactttgactattgggggcagggaactctggtcaccgtgagctccgcctccaccaagggaccttctgtgttcccactggctccctctagtaaatccacatctgggggaactgcagccctgggctgtctggtgaagggctacttcccagagcccgtcacagtgtcttggaacagtggcgctctgacttctggggtccacacctttcctgcagtgctgaagtcaagcgggctgtacagcctgtcctctgtggtcaccgtgccaagttcaagcctgggaacacagacttatatctgcaacgtgaatcacaagccatccaatacaaaagtcgacaagaaagtggaacccaagtcttgtgataaaacccatacatgccccccttgtcctgcaccagagctgctgggaggaccaagcgtgttcctgtttccacccaagcctaaagatacactgatgattagtaggaccccagaagtcacatgcgtggtcgtggacgtgagccacgaggaccccgaagtcaagtttaactggtacgtggacggcgtcgaggtgcataatgccaagactaaacccagggaggaacagtacaacagtacctatcgcgtcgtgtcagtcctgacagtgctgcatcaggattggctgaacgggaaagagtataagtgcaaagtgagcaataaggctctgcccgcacctatcgagaaaacaatttccaaggcaaaaggacagcctagagaaccacaggtgtacgtgctgcctccatcaagggatgagctgacaaagaaccaggtcagcctgctgtgtctggtgaaaggattctatccctctgacattgctgtggagtgggaaagtaatggccagcctgagaacaattacctgacctggccccctgtgctggactcagatggcagcttctttctgtatagcaagctgaccgtcgacaaatcccggtggcagcaggggaatgtgtttagttgttcagtcatgcacgaggcactgcacaaccattacacccagaagtcactgtcactgtcaccaggg

SEQ ID NO: 5 - protein, 119 aa, Artificial Sequence [sequence omitted]

SEQ ID NO: 6 - protein, 8 aa, Artificial Sequence
  Artificial sequence
GFTFTDYT

SEQ ID NO: 7 - protein, 12 aa, Artificial Sequence
  Artificial sequence
ARNLGPSFYFDY

SEQ ID NO: 8 - protein, 8 aa, Artificial Sequence
  Artificial sequence
VNPNSGGS

SEQ ID NO: 9 - protein, 214 aa, Artificial Sequence
  Artificial sequence
DIQMTQSPSSLSASVGDRVTITCKASQDVSIGVAWYQQKPGKAPKLLIYSASYRYTGVPSRFSGSGSGTDFTLTISSLQPEDFATYYCQQYYIYPYTFGQGTKVEIKRTVAAPSVFIFPPSDEQLKSGTASVVCLLNNFYPREAKVQWKVDNALQSGNSQESVTEQDSKDSTYSLSSTLTLSKADYEKHKVYACEVTHQGLSSPVTKSFNRGEC

SEQ ID NO: 10 - DNA, 642 bp, Artificial Sequence
  Artificial sequence
gatattcagatgacccagtccccaagctccctgagtgcctcagtgggcgaccgagtcaccatcacatgcaaggcttcccaggatgtgtctattggagtcgcatggtaccagcagaagccaggcaaagcacccaagctgctgatctatagcgcctcctaccggtataccggcgtgccctctagattctctggcagtgggtcaggaacagactttactctgaccatctctagtctgcagcctgaggatttcgctacctactattgccagcagtactatatctacccatatacctttggccaggggacaaaagtggagatcaagaggactgtggccgctccctccgtcttcatttttcccccttctgacgaacagctgaaaagtggcacagccagcgtggtctgtctgctgaacaatttctaccctcgcgaagccaaagtgcagtggaaggtcgataacgctctgcagagcggcaacagccaggagtctgtgactgaacaggacagtaaagattcaacctatagcctgtcaagcacactgactctgagcaaggcagactacgagaagcacaaagtgtatgcctgcgaagtcacacatcaggggctgtcctctcctgtgactaagagctttaacagaggagagtgt

SEQ ID NO: 11 - protein, 107 aa, Artificial Sequence [sequence omitted]

SEQ ID NO: 12 - protein, 6 aa, Artificial sequence
  Artificial sequence
QDVSIG

SEQ ID NO: 13 - protein, 9 aa, Artificial Sequence
  Artificial sequence
QQYYIYPYT

SEQ ID NO: 14 - protein, 3 aa, Artificial Sequence
  Artificial sequence
SAS

SEQ ID NO: 15 - protein, 222 aa, Artificial Sequence
  Artificial sequence
DYKDDDDKDIQMTQSPSSLSASVGDRVTITCRASQDVNTAVAWYQQKPGKAPKLLIYSASFLYSGVPSRFSGSRSGTDFTLTISSLQPEDFATYYCQQHYTTPPTFGQGTKVEIKRTVAAPSVFIFPPSDERLKSGTASVVCLLNNFYPREAKVQWKVDNALQSGNSQESVTEQDSKDSTYSLSSTLTLSKADYEKHKVYACEVTHQGLSSPVTKSFNRGEC

SEQ ID NO: 16 - DNA, 666 bp, Artificial Sequence
  Artificial sequence
gactacaaagacgacgatgacaaagatatccagatgacccagtcccctagctccctgtccgcttctgtgggcgatagggtcactattacctgccgcgcatctcaggacgtgaacaccgcagtcgcctggtaccagcagaagcctgggaaagctccaaagctgctgatctacagtgcatcattcctgtattcaggagtgcccagccggtttagcggcagcagatctggcaccgatttcacactgactatttctagtctgcagcctgaggactttgccacatactattgccagcagcactataccacaccccctactttcggccaggggaccaaagtggagatcaagcgaactgtggccgctccaagtgtcttcatttttccacccagcgatgaaagactgaagtccggcacagcttctgtggtctgtctgctgaacaatttttaccccagagaggccaaagtgcagtggaaggtcgacaacgctctgcagagtggcaacagccaggagagcgtgacagaacaggattccaaagactctacttatagtctgtcaagcaccctgacactgagcaaggcagactacgaaaagcataaagtgtatgcctgtgaggtcacacatcaggggctgtcatcaccagtcaccaaatcattcaatcggggggagtgc

SEQ ID NO: 17 - protein, 107 aa, Artificial Sequence [sequence omitted]

SEQ ID NO: 18 - protein, 222 aa, Artificial Sequence
  Artificial sequence
DYKDDDDKDIQMTQSPSSLSASVGDRVTITCRASQDVNTAVAWYQQKPGKAPKLLIYSASFLYSGVPSRFSGSRSGTDFTLTISSLQPEDFATYYCQQHYTTPPTFGQGTKVEIKRTVAAPSVFIFPPSDERLKSGTASVVCLLNNFYPREAKVQWKVDNALQSGNSKESVTEQDSKDSTYSLSSRLTLSKADYEKHKVYACEVTHQGLSSPVTKSFNRGEC

SEQ ID NO: 19 - DNA, 666 bp, Artificial Sequence
  Artificial sequence
gactacaaagacgacgatgacaaagatatccagatgacccagtcccctagctccctgtccgcttctgtgggcgatagggtcactattacctgccgcgcatctcaggacgtgaacaccgcagtcgcctggtaccagcagaagcctgggaaagctccaaagctgctgatctacagtgcatcattcctgtattcaggagtgcccagccggtttagcggcagcagatctggcaccgatttcacactgactatttctagtctgcagcctgaggactttgccacatactattgccagcagcactataccacaccccctactttcggccaggggaccaaagtggagatcaagcgaactgtggccgctccaagtgtcttcatttttccacccagcgatgaaagactgaagtccggcacagcttctgtggtctgtctgctgaacaatttttaccccagagaggccaaagtgcagtggaaggtcgacaacgctctgcagagtggcaacagcaaggagagcgtgacagaacaggattccaaagactctacttatagtctgtcaagcagactgacactgagcaaggcagactacgaaaagcataaagtgtatgcctgtgaggtcacacatcaggggctgtcatcaccagtcaccaaatcattcaatcggggggagtgc

SEQ ID NO: 20 - protein, 107 aa, Artificial Sequence [sequence omitted]

SEQ ID NO: 21 - protein, 6 aa, Artificial Sequence
  Artificial sequence
QDVNTA

SEQ ID NO: 22 - protein, 9 aa, Artificial Sequence
  Artificial sequence
QQHYTTPPT

SEQ ID NO: 23 - protein, 3 aa, Artificial Sequence
  Artificial sequence
SAS

SEQ ID NO: 24 - protein, 214 aa, Artificial Sequence
  Artificial sequence
DIQMTQSPSSLSASVGDRVTITCKASQDVSIGVAWYQQKPGKAPKLLIYSASYRYTGVPSRFSGSGSGTDFTLTISSLQPEDFATYYCQQYYIYPATFGQGTKVEIKRTVAAPSVFIFPPSDEQLKSGTASVVCLLNNFYPREAKVQWKVDNALQSGNSQESVTEQDSKDSTYSLSSTLTLSKADYEKHKVYACEVTHQGLSSPVTKSFNRGEC

SEQ ID NO: 25 - DNA, 642 bp, Artificial Sequence
  Artificial sequence
gatattcagatgacccagtccccaagctccctgagtgcctcagtgggcgaccgagtcaccatcacatgcaaggcttcccaggatgtgtctattggagtcgcatggtaccagcagaagccaggcaaagcacccaagctgctgatctatagcgcctcctaccggtataccggcgtgccctctagattctctggcagtgggtcaggaacagactttactctgaccatctctagtctgcagcctgaggatttcgctacctactattgccagcagtactatatctacccagccacctttggccaggggacaaaagtggagatcaagaggactgtggccgctccctccgtcttcatttttcccccttctgacgaacagctgaaaagtggcacagccagcgtggtctgtctgctgaacaatttctaccctcgcgaagccaaagtgcagtggaaggtcgataacgctctgcagagcggcaacagccaggagtctgtgactgaacaggacagtaaagattcaacctatagcctgtcaagcacactgactctgagcaaggcagactacgagaagcacaaagtgtatgcctgcgaagtcacacatcaggggctgtcctctcctgtgactaagagctttaacagaggagagtgt

SEQ ID NO: 26 - protein, 107 aa, Artificial Sequence
  Artificial sequence
DIQMTQSPSSLSASVGDRVTITCKASQDVSIGVAWYQQKPGKAPKLLIYSASYRYTGVPSRFSGSGSGTDFTLTISSLQPEDFATYYCQQYYIYPATFGQGTKVEIK

SEQ ID NO: 27 - protein, 6 aa, Artificial Sequence
  Artificial sequence
QDVSIG

SEQ ID NO: 28 - protein, 9 aa, Artificial Sequence
  Artificial sequence
QQYYIYPAT

SEQ ID NO: 29 - protein, 3 aa, Artificial Sequence
  Artificial sequence
SAS

SEQ ID NO: 30 - protein, 449 aa, Artificial Sequence
  Artificial sequence
EVQLVESGGGLVQPGGSLRLSCAASGFNIKDTYIHWVRQAPGKGLEWVARIYPTNGYTRYADSVKGRFTISADTSKNTAYLQMNSLRAEDTAVYYCSRWGGDGFYAMDYWGQGTLVTVSSASTKGPSVFPLAPSSKSTSGGTAALGCEVTDYFPEPVTVSWNSGALTSGVHTFPAVLQSSGLYSLSSVVTVPSSSLGTQTYICNVNHKPSNTKVDKKVEPKSCDKTHTCPPCPAPELLGGPSVFLFPPKPKDTLMISRTPEVTCVVVDVSHEDPEVKFNWYVDGVEVHNAKTKPREEQYNSTYRVVSVLTVLHQDWLNGKEYKCKVSNKALPAPIEKTISKAKGQPREPQVYVYPPSRDELTKNQVSLTCLVKGFYPSDIAVEWESNGQPENNYKTTPPVLDSDGSFALVSKLTVDKSRWQQGNVFSCSVMHEALHNHYTQKSLSLSPG

SEQ ID NO: 31 - DNA, 1347 bp, Artificial Sequence
  Artificial sequence
gaggtgcagctggtcgaaagcggaggaggactggtgcagccaggagggtcactgcgactgagctgcgcagcttccggcttcaacatcaaggacacctacattcactgggtccgccaggctcctggaaaaggcctggagtgggtggcacgaatctatccaactaatggatacacccggtatgccgactccgtgaagggccggttcaccatttctgcagatacaagtaaaaacactgcctacctgcagatgaacagcctgcgagccgaagatacagccgtgtactattgcagccgatggggaggcgacggcttctacgctatggattattgggggcagggaaccctggtcacagtgagctccgcatcaacaaaggggcctagcgtgtttccactggccccctctagtaaatccacctctgggggaacagcagccctgggatgtgaggtgaccgactacttcccagagcccgtcactgtgagctggaactccggcgccctgacatctggggtccatacttttcctgctgtgctgcagtcaagcggcctgtacagcctgtcctctgtggtcactgtgccaagttcaagcctggggactcagacctatatctgcaacgtgaatcacaagccatccaataccaaagtcgacaagaaagtggaacccaagtcttgtgataaaacacatacttgccccccttgtcctgcaccagagctgctgggaggaccaagcgtgttcctgtttccacccaagcctaaagacaccctgatgattagtaggactccagaagtcacctgcgtggtcgtggacgtgagccacgaggaccccgaagtcaagttcaactggtacgtggatggcgtcgaggtgcataatgccaagacaaaacccagggaggaacagtacaactccacttatcgcgtcgtgtctgtcctgaccgtgctgcaccaggactggctgaacggcaaggagtataagtgcaaagtgagcaataaggctctgcccgcacctatcgagaaaacaatttccaaggctaaagggcagcctagagaaccacaggtgtacgtgtaccctccatctagggacgagctgaccaagaaccaggtcagtctgacatgtctggtgaaagggttctatcccagcgatatcgcagtggagtgggaatccaatggacagcctgagaacaattacaagaccacaccccctgtgctggactctgatggaagtttcgccctggtgagtaagctgaccgtcgataaatcacggtggcagcagggcaacgtgttcagctgttcagtgatgcacgaagcactgcacaaccactacacccagaaaagcctgtccctgtcccccggc

SEQ ID NO: 32 - protein, 120 aa, Artificial Sequence [sequence omitted]

SEQ ID NO: 33 - protein, 8 aa, Artificial Sequence
  Artificial sequence
GFNIKDTY

SEQ ID NO: 34 - protein, 13 aa, Artificial Sequence
  Artificial sequence
SRWGGDGFYAMDY

SEQ ID NO: 35 - protein, 8 aa, Artificial Sequence
  Artificial sequence
IYPTNGYT

SEQ ID NO: 36 - protein, 448 aa, Artificial Sequence
  Artificial sequence
EVQLVESGGGLVQPGGSLRLSCAASGFTFADYTMDWVRQAPGKGLEWVGDVNPNSGGSIYNQRFKGRFTFSVDRSKNTLYLQMNSLRAEDTAVYYCARNLGPSFYFDYWGQGTLVTVSSASTKGPSVFPLAPSSKSTSGGTAALGCLVKDYFPEPVTVSWNSGALTSGVHTFPAVLQSSGLYSLSSVVTVPSSSLGTQTYICNVNHKPSNTKVDKKVEPKSCDKTHTCPPCPAPELLGGPSVFLFPPKPKDTLMISRTPEVTCVVVDVSHEDPEVKFNWYVDGVEVHNAKTKPREEQYNSTYRVVSVLTVLHQDWLNGKEYKCKVSNKALPAPIEKTISKAKGQPREPQVYVYPPSRDELTKNQVSLTCLVKGFYPSDIAVEWESNGQPENNYKTTPPVLDSDGSFALVSKLTVDKSRWQQGNVFSCSVMHEALHNHYTQKSLSLSPG

SEQ ID NO: 37 - DNA, 1344 bp, Artificial Sequence
  Artificial sequence
gaggtgcagctggtggaatcaggagggggcctggtgcagcccggagggtctctgcgactgtcatgtgccgcttctgggttcactttcgcagactacacaatggattgggtgcgacaggcccccggaaagggactggagtgggtgggcgatgtcaaccctaattctggcgggagtatctacaaccagcggttcaaggggagattcactttttcagtggacagaagcaaaaacaccctgtatctgcagatgaacagcctgagggccgaagataccgctgtctactattgcgctcgcaatctgggccccagtttctactttgactattgggggcagggaaccctggtgacagtcagctccgctagcactaaggggccttccgtgtttccactggctccctctagtaaatccacctctggaggcacagctgcactgggatgtctggtgaaggattacttccctgaaccagtcacagtgagttggaactcaggggctctgacaagtggagtccatacttttcccgcagtgctgcagtcaagcggactgtactccctgtcctctgtggtcaccgtgcctagttcaagcctgggcacccagacatatatctgcaacgtgaatcacaagccatcaaatacaaaagtcgacaagaaagtggagcccaagagctgtgataaaactcatacctgcccaccttgtccggcgccagaactgctgggaggaccaagcgtgttcctgtttccacccaagcctaaagacaccctgatgatttcccggactcctgaggtcacctgcgtggtcgtggacgtgtctcacgaggaccccgaagtcaagttcaactggtacgtggatggcgtcgaagtgcataatgccaagaccaaaccccgggaggaacagtacaactctacctatagagtcgtgagtgtcctgacagtgctgcaccaggactggctgaatgggaaggagtataagtgtaaagtgagcaacaaagccctgcccgccccaatcgaaaaaacaatctctaaagcaaaaggacagcctcgcgaaccacaggtctacgtctaccccccatcaagagatgaactgacaaaaaatcaggtctctctgacatgcctggtcaaaggattctacccttccgacatcgccgtggagtgggaaagtaacggccagcccgagaacaattacaagaccacaccccctgtcctggactctgatgggagtttcgctctggtgtcaaagctgaccgtcgataaaagccggtggcagcagggcaatgtgtttagctgctccgtcatgcacgaagccctgcacaatcactacacacagaagtccctgagcctgagccctggc

SEQ ID NO: 38 - protein, 119 aa, Artificial Sequence
  Artificial sequence
EVQLVESGGGLVQPGGSLRLSCAASGFTFADYTMDWVRQAPGKGLEWVGDVNPNSGGSIYNQRFKGRFTFSVDRSKNTLYLQMNSLRAEDTAVYYCARNLGPSFYFDYWGQGTLVTVSS

SEQ ID NO: 39 - protein, 8 aa, Artificial Sequence
  Artificial sequence
GFTFADYT

SEQ ID NO: 40 - protein, 12 aa, Artificial Sequence
  Artificial sequence
ARNLGPSFYFDY

SEQ ID NO: 41 - protein, 8 aa, Artificial Sequence
  Artificial sequence
VNPNSGGS

SEQ ID NO: 42 - protein, 226 aa, Artificial Sequence
  Artifcial sequence
YPYDVPDYATGSDIQMTQSPSSLSASVGDRVTITCKASQDVSIGVAWYQQKPGKAPKLLIYSASYRYTGVPSRFSGSGSGTDFTLTISSLQPEDFATYYCQQYYIYPYTFGQGTKVEIKRTVAAPSVFIFPPSDEELKSGTASVVCLLNNFYPREAKVQWKVDNALQSGNSEESVTEQDSKDSTYSLSSTLELSKADYEKHKVYACEVTHQGLSSPVTKSFNRGEC

SEQ ID NO: 43 - DNA, 678 bp, Artificial Sequence
  Artificial sequence
tatccctacgatgtgcctgactacgctactggctccgatatccagatgacccagtctccaagctccctgagtgcatcagtgggggaccgagtcaccatcacatgcaaggcttcccaggatgtgtctattggagtcgcatggtaccagcagaagccaggcaaagcacccaagctgctgatctacagcgcctcctaccggtatactggggtgccttccagattctctggcagtgggtcaggaaccgactttactctgaccatctctagtctgcagcccgaggatttcgccacctactattgccagcagtactatatctacccttatacctttggccaggggacaaaagtggagatcaagaggacagtggccgctccaagtgtcttcatttttcccccttccgacgaagagctgaaaagtggaactgcttcagtggtctgtctgctgaacaatttctacccccgcgaagccaaagtgcagtggaaggtcgataacgctctgcagagcggcaattccgaggagtctgtgacagaacaggacagtaaagattcaacttatagcctgtcaagcacactggagctgtctaaggcagactacgagaagcacaaagtgtatgcctgcgaagtcacccatcaggggctgtcctctcccgtgacaaagagctttaacagaggagagtgt

SEQ ID NO: 44 - protein, 107 aa, Artificial Sequence [sequence omitted]

SEQ ID NO: 45 - protein, 481 aa, Artificial Sequence
  Artificial sequence
DIQMTQSPSSLSASVGDRVTITCRASQDVNTAVAWYQQKPGKAPKLLIYSASFLYSGVPSRFSGSRSGTDFTLTISSLQPEDFATYYCQQHYTTPPTFGQGTKVEIKGGSGGGSGGGSGGGSGGGSGEVQLVESGGGLVQPGGSLRLSCAASGFNIKDTYIHWVRQAPGKGLEWVARIYPTNGYTRYADSVKGRFTISADTSKNTAYLQMNSLRAEDTAVYYCSRWGGDGFYAMDYWGQGTLVTVSSAAEPKSSDKTHTCPPCPAPELLGGPSVFLFPPKPKDTLMISRTPEVTCVVVDVSHEDPEVKFNWYVDGVEVHNAKTKPREEQYNSTYRVVSVLTVLHQDWLNGKEYKCKVSNKALPAPIEKTISKAKGQPREPQVYTYPPSRDELTKNQVSLTCLVKGFYPSDIAVEWESNGQPENNYKTTPPVLDEDGSFALVSKLTVDKSRWQQGNVFSCSVMHEALHNHYTQKSLSLSPGK

SEQ ID NO: 46 - DNA, 1443 bp, Artificial Sequence
  Artificial sequence
gacatccagatgacccagtctccatcctccctgtctgcatctgtaggagacagagtcaccatcacttgccgggcaagtcaggacgttaacaccgctgtagcttggtatcagcagaaaccagggaaagcccctaagctcctgatctattctgcatcctttttgtacagtggggtcccatcaaggttcagtggcagtcgatctgggacagatttcactctcaccatcagcagtctgcaacctgaagattttgcaacttactactgtcaacagcattacactaccccacccactttcggccaagggaccaaagtggagatcaaaggtggttctggtggtggttctggtggtggttctggtggtggttctggtggtggttctggtgaagtgcagctggtggagtctgggggaggcttggtacagcctggcgggtccctgagactctcctgtgcagcctctggattcaacattaaagatacttatatccactgggtccggcaagctccagggaagggcctggagtgggtcgcacgtatttatcccacaaatggttacacacggtatgcggactctgtgaagggccgattcaccatctccgcagacacttccaagaacaccgcgtatctgcaaatgaacagtctgagagctgaggacacggccgtttattactgttcaagatggggcggagacggtttctacgctatggactactggggccaagggaccctggtcaccgtctcctcagccgccgagcccaagagcagcgataagacccacacctgccctccctgtccagctccagaactgctgggaggacctagcgtgttcctgtttccccctaagccaaaagacactctgatgatttccaggactcccgaggtgacctgcgtggtggtggacgtgtctcacgaggaccccgaagtgaagttcaactggtacgtggatggcgtggaagtgcataatgctaagacaaaaccaagagaggaacagtacaactccacttatcgcgtcgtgagcgtgctgaccgtgctgcaccaggactggctgaacgggaaggagtataagtgcaaagtcagtaataaggccctgcctgctccaatcgaaaaaaccatctctaaggccaaaggccagccaagggagccccaggtgtacacatacccacccagcagagacgaactgaccaagaaccaggtgtccctgacatgtctggtgaaaggcttctatcctagtgatattgctgtggagtgggaatcaaatggacagccagagaacaattacaagaccacacctccagtgctggacgaggatggcagcttcgccctggtgtccaagctgacagtggataaatctcgatggcagcaggggaacgtgtttagttgttcagtgatgcatgaagccctgcacaatcattacactcagaagagcctgtccctgtctcccggcaaa

SEQ ID NO: 47 - protein, 107 aa, Artificial Sequence [sequence omitted]

SEQ ID NO: 48 - protein, 120 aa, Artificial Sequence [sequence omitted]

SEQ ID NO: 49 - protein, 481 aa, Artificial Sequence
  Artificial sequence
DIQMTQSPSSLSASVGDRVTITCRASQDVNTAVAWYQQKPGKAPKLLIYSASFLYSGVPSRFSGSRSGTDFTLTISSLQPEDFATYYCQQHYTTPPTFGQGTKVEIKGGSGGGSGGGSGGGSGGGSGEVQLVESGGGLVQPGGSLRLSCAASGFNIKDTYIHWVRQAPGKGLEWVARIYPTNGYTRYADSVKGRFTISADTSKNTAYLQMNSLRAEDTAVYYCSRWGGDGFYAMDYWGQGTLVTVSSAAEPKSSDKTHTCPPCPAPELLGGPSVFLFPPKPKDTLMISRTPEVTCVVVDVSHEDPEVKFNWYVDGVEVHNAKTKPREEQYNSTYRVVSVLTVLHQDWLNGKEYKCKVSNKALPAPIEKTISKAKGQPREPQVYTLPPSRDELTKNQVSLICLVKGFYPSDIAVEWESNGQPENRYMTWPPVLDSDGSFFLYSKLTVDKSRWQQGNVFSCSVMHEALHNHYTQKSLSLSPGK

SEQ ID NO: 50 - DNA, 1443 bp, Artificial Sequence
  Artificial sequence
gacatccagatgacccagtctccatcctccctgtctgcatctgtaggagacagagtcaccatcacttgccgggcaagtcaggacgttaacaccgctgtagcttggtatcagcagaaaccagggaaagcccctaagctcctgatctattctgcatcctttttgtacagtggggtcccatcaaggttcagtggcagtcgatctgggacagatttcactctcaccatcagcagtctgcaacctgaagattttgcaacttactactgtcaacagcattacactaccccacccactttcggccaagggaccaaagtggagatcaaaggtggttctggtggtggttctggtggtggttctggtggtggttctggtggtggttctggtgaagtgcagctggtggagtctgggggaggcttggtacagcctggcgggtccctgagactctcctgtgcagcctctggattcaacattaaagatacttatatccactgggtccggcaagctccagggaagggcctggagtgggtcgcacgtatttatcccacaaatggttacacacggtatgcggactctgtgaagggccgattcaccatctccgcagacacttccaagaacaccgcgtatctgcaaatgaacagtctgagagctgaggacacggccgtttattactgttcaagatggggcggagacggtttctacgctatggactactggggccaagggaccctggtcaccgtctcctcagccgccgagcccaagagcagcgataagacccacacctgccctccctgtccagctccagaactgctgggaggacctagcgtgttcctgtttccccctaagccaaaagacactctgatgatttccaggactcccgaggtgacctgcgtggtggtggacgtgtctcacgaggaccccgaagtgaagttcaactggtacgtggatggcgtggaagtgcataatgctaagacaaaaccaagagaggaacagtacaactccacttatcgcgtcgtgagcgtgctgaccgtgctgcaccaggactggctgaacgggaaggagtataagtgcaaagtcagtaataaggccctgcctgctccaatcgaaaaaaccatctctaaggccaaaggccagccaagggagccccaggtgtacacactgccacccagcagagacgaactgaccaagaaccaggtgtccctgatctgtctggtgaaaggcttctatcctagtgatattgctgtggagtgggaatcaaatggacagccagagaacagatacatgacctggcctccagtgctggacagcgatggcagcttcttcctgtattccaagctgacagtggataaatctcgatggcagcaggggaacgtgtttagttgttcagtgatgcatgaagccctgcacaatcattacactcagaagagcctgtccctgtctcccggcaaa

SEQ ID NO: 51 - protein, 107 aa, Artificial Sequence [sequence omitted]

SEQ ID NO: 52 - protein, 120 aa, Artificial Sequence [sequence omitted]

SEQ ID NO: 53 - protein, 448 aa, Artificial Sequence
  Artificial sequence
EVQLVESGGGLVQPGGSLRLSCAASGFTFTDYTMDWVRQAPGKGLEWVADVNPNSGGSIYNQRFKGRFTLSVDRSKNTLYLQMNSLRAEDTAVYYCARNLGPSFYFDYWGQGTLVTVSSASTKGPSVFPLAPSSKSTSGGTAALGCLVKDYFPEPVTVSWNSGALTSGVHTFPAVLQSSGLYSLSSVVTVPSSSLGTQTYICNVNHKPSNTKVDKKVEPKSCDKTHTCPPCPAPELLGGPSVFLFPPKPKDTLMISRTPEVTCVVVDVSHEDPEVKFNWYVDGVEVHNAKTKPREEQYNSTYRVVSVLTVLHQDWLNGKEYKCKVSNKALPAPIEKTISKAKGQPREPQVYVLPPSRDELTKNQVSLLCLVKGFYPSDIAVEWESNGQPENNYLTWPPVLDSDGSFFLYSKLTVDKSRWQQGNVFSCSVMHEALHNHYTQKSLSLSPG

SEQ ID NO: 54 - DNA, 1344 bp, Artificial Sequence
  Artificial sequence
gaagtgcagctggtcgaatctggaggaggactggtgcagccaggagggtccctgcgcctgtcttgcgccgctagtggcttcacttttaccgactacaccatggattgggtgcgacaggcacctggaaagggcctggagtgggtcgccgatgtgaacccaaatagcggaggctccatctacaaccagcggttcaagggccggttcaccctgtcagtggaccggagcaaaaacaccctgtatctgcagatgaatagcctgcgagccgaagatactgctgtgtactattgcgcccggaatctggggccctccttctactttgactattgggggcagggaactctggtcaccgtgagctccgcctccaccaagggaccttctgtgttcccactggctccctctagtaaatccacatctgggggaactgcagccctgggctgtctggtgaaggactacttcccagagcccgtcacagtgtcttggaacagtggcgctctgacttctggggtccacacctttcctgcagtgctgcagtcaagcgggctgtacagcctgtcctctgtggtcaccgtgccaagttcaagcctgggaacacagacttatatctgcaacgtgaatcacaagccatccaatacaaaagtcgacaagaaagtggaacccaagtcttgtgataaaacccatacatgccccccttgtcctgcaccagagctgctgggaggaccaagcgtgttcctgtttccacccaagcctaaagatacactgatgattagtaggaccccagaagtcacatgcgtggtcgtggacgtgagccacgaggaccccgaagtcaagtttaactggtacgtggacggcgtcgaggtgcataatgccaagactaaacccagggaggaacagtacaacagtacctatcgcgtcgtgtcagtcctgacagtgctgcatcaggattggctgaacgggaaagagtataagtgcaaagtgagcaataaggctctgcccgcacctatcgagaaaacaatttccaaggcaaaaggacagcctagagaaccacaggtgtacgtgctgcctccatcaagggatgagctgacaaagaaccaggtcagcctgctgtgtctggtgaaaggattctatccctctgacattgctgtggagtgggaaagtaatggccagcctgagaacaattacctgacctggccccctgtgctggactcagatggcagcttctttctgtatagcaagctgaccgtcgacaaatcccggtggcagcaggggaatgtgtttagttgttcagtcatgcacgaggcactgcacaaccattacacccagaagtcactgtcactgtcaccaggg

SEQ ID NO: 55 - protein, 119 aa, Artificial Sequence [sequence omitted]

SEQ ID NO: 56 - protein, 448 aa, Artificial Sequence
  Artificial sequence
EVQLVESGGGLVQPGGSLRLSCAASGFTFTDYTMDWVRQAPGKGLEWVADVNPNSGGSIYNQRFKGRFTLSVDRSKNTLYLQMNSLRAEDTAVYYCARNLGPSFYFDYWGQGTLVTVSSASTKGPSVFPLAPSSKSTSGGTAALGCLVKDYFPEPVTVSWNSGALTSGVHTFPAVLQSSGLYSLSSVVTVPSSSLGTQTYICNVNHKPSNTKVDKKVEPKSCDKTHTCPPCPAPELLGGPSVFLFPPKPKDTLMISRTPEVTCVVVDVSHEDPEVKFNWYVDGVEVHNAKTKPREEQYNSTYRVVSVLTVLHQDWLNGKEYKCKVSNKALPAPIEKTISKAKGQPREPQVYVYPPSRDELTKNQVSLTCLVKGFYPSDIAVEWESNGQPENNYKTTPPVLDSDGSFALVSKLTVDKSRWQQGNVFSCSVMHEALHNHYTQKSLSLSPG

SEQ ID NO: 57 - DNA, 1344 bp, Artificial Sequence
  Artificial sequence
gaagtgcagctggtcgaatctggaggaggactggtgcagccaggagggtccctgcgcctgtcttgcgccgctagtggcttcacttttaccgactacaccatggattgggtgcgacaggcacctggaaagggcctggagtgggtcgccgatgtgaacccaaatagcggaggctccatctacaaccagcggttcaagggccggttcaccctgtcagtggaccggagcaaaaacaccctgtatctgcagatgaatagcctgcgagccgaagatactgctgtgtactattgcgcccggaatctggggccctccttctactttgactattgggggcagggaactctggtcaccgtgagctccgcctccaccaagggaccttctgtgttcccactggctccctctagtaaatccacatctgggggaactgcagccctgggctgtctggtgaaggactacttcccagagcccgtcacagtgtcttggaacagtggcgctctgacttctggggtccacacctttcctgcagtgctgcagtcaagcgggctgtacagcctgtcctctgtggtcaccgtgccaagttcaagcctgggaacacagacttatatctgcaacgtgaatcacaagccatccaatacaaaagtcgacaagaaagtggaacccaagtcttgtgataaaacccatacatgccccccttgtcctgcaccagagctgctgggaggaccaagcgtgttcctgtttccacccaagcctaaagatacactgatgattagtaggaccccagaagtcacatgcgtggtcgtggacgtgagccacgaggaccccgaagtcaagtttaactggtacgtggacggcgtcgaggtgcataatgccaagactaaacccagggaggaacagtacaacagtacctatcgcgtcgtgtcagtcctgacagtgctgcatcaggattggctgaacgggaaagagtataagtgcaaagtgagcaataaggctctgcccgcacctatcgagaaaacaatttccaaggcaaaaggacagcctagagaaccacaggtgtacgtgtatcctccatcaagggatgagctgacaaagaaccaggtcagcctgacttgtctggtgaaaggattctatccctctgacattgctgtggagtgggaaagtaatggccagcctgagaacaattacaagaccacaccccctgtgctggactcagatggcagcttcgcgctggtgagcaagctgaccgtcgacaaatcccggtggcagcaggggaatgtgtttagttgttcagtcatgcacgaggcactgcacaaccattacacccagaagtcactgtcactgtcaccaggg

SEQ ID NO: 58 - protein, 119 aa, Artificial Sequence [sequence omitted]

SEQ ID NO: 59 - protein, 475 aa, Artificial Sequence
  Artificial sequence
DIQMTQSPSSLSASVGDRVTITCKASQDVSIGVAWYQQKPGKAPKLLIYSASYRYTGVPSRFSGSGSGTDFTLTISSLQPEDFATYYCQQYYIYPYTFGQGTKVEIKGGGGSGGGGSGGGGSEVQLVESGGGLVQPGGSLRLSCAASGFTFTDYTMDWVRQAPGKGLEWVADVNPNSGGSIYNQRFKGRFTLSVDRSKNTLYLQMNSLRAEDTAVYYCARNLGPSFYFDYWGQGTLVTVSSAAEPKSSDKTHTCPPCPAPELLGGPSVFLFPPKPKDTLMISRTPEVTCVVVDVSHEDPEVKFNWYVDGVEVHNAKTKPREEQYNSTYRVVSVLTVLHQDWLNGKEYKCKVSNKALPAPIEKTISKAKGQPREPQVYVYPPSRDELTKNQVSLTCLVKGFYPSDIAVEWESNGQPENNYKTTPPVLDSDGSFALVSKLTVDKSRWQQGNVFSCSVMHEALHNHYTQKSLSLSPGK

SEQ ID NO: 60 - DNA, 1425 bp, Artificial Sequence
  Artificial sequence
gacattcagatgacccagagccctagctccctgagtgcctcagtcggggacagggtgactatcacctgcaaggcttcacaggatgtcagcattggcgtggcatggtaccagcagaagccagggaaagcacccaagctgctgatctatagcgcctcctacaggtatacaggcgtgccatcccgcttctctggcagtgggtcaggaactgactttacactgactatttctagtctgcagcccgaagatttcgccacatactattgccagcagtactatatctacccttatacttttggccaggggaccaaagtggagattaagggcggaggaggctccggaggaggagggtctggaggaggaggaagtgaggtccagctggtggaatctggaggaggactggtgcagccaggagggtccctgaggctgtcttgtgccgctagtggcttcacctttacagactacacaatggattgggtgcgccaggcaccaggaaagggactggaatgggtcgctgatgtgaaccctaatagcggaggctccatctacaaccagcggttcaaaggacggttcaccctgtcagtggaccggagcaagaacaccctgtatctgcagatgaacagcctgagagccgaggatactgctgtgtactattgcgccaggaatctgggcccaagcttctactttgactattgggggcagggaacactggtcactgtgtcaagcgcagccgaacccaaatcctctgataagactcacacctgcccaccttgtccagctccagagctgctgggaggacctagcgtgttcctgtttccacccaagccaaaagacactctgatgatttctagaacccctgaagtgacatgtgtggtcgtggacgtcagtcacgaggaccccgaagtcaaattcaactggtacgtggatggcgtcgaggtgcataatgccaagaccaaaccccgagaggaacagtacaactcaacctatcgggtcgtgagcgtcctgacagtgctgcatcaggactggctgaacggcaaggagtataagtgcaaagtgagcaacaaggctctgcctgcaccaatcgagaagaccatttccaaggctaaagggcagccccgcgaacctcaggtctacgtgtatcctccaagccgagatgagctgacaaaaaaccaggtctccctgacttgtctggtgaagggattttacccaagtgacatcgcagtggagtgggaatcaaatggccagcccgaaaacaattataagaccacaccccctgtgctggactctgatgggagtttcgcactggtctccaaactgaccgtggacaagtctcggtggcagcagggaaacgtctttagctgttccgtgatgcacgaggccctgcacaatcattacacacagaaatctctgagtctgtcacctggcaag

SEQ ID NO: 61 - protein, 107 aa, Artificial Sequence [sequence omitted]

SEQ ID NO: 62 - protein, 119 aa, Artificial Sequence [sequence omitted]

SEQ ID NO: 63 - protein, 480 aa, Artificial Sequence
  Artificial sequence
DIQMTQSPSSLSASVGDRVTITCRASQDVNTAVAWYQQKPGKAPKLLIYSASFLYSGVPSRFSGSRSGTDFTLTISSLQPEDFATYYCQQHYTTPPTFGQGTKVEIKGGSGGGSGGGSGGGSGGGSGEVQLVESGGGLVQPGGSLRLSCAASGFNIKDTYIHWVRQAPGKGLEWVARIYPTNGYTRYADSVKGRFTISADTSKNTAYLQMNSLRAEDTAVYYCSRWGGDGFYAMDYWGQGTLVTVSSAAEPKSSDKTHTCPPCPAPELLGGPSVFLFPPKPKDTLMISRTPEVTCVVVDVSHEDPEVKFNWYVDGVEVHNAKTKPREEQYNSTYRVVSVLTVLHQDWLNGKEYKCKVSNKALPAPIEKTISKAKGQPREPQVYVLPPSRDELTKNQVSLLCLVKGFYPSDIAVEWESNGQPENNYLTWPPVLDSDGSFFLYSKLTVDKSRWQQGNVFSCSVMHEALHNHYTQKSLSLSPG

SEQ ID NO: 64 - DNA, 1440 bp, Artificial Sequence
  Artificial sequence
gacattcagatgacacagagccccagctccctgagtgcttcagtcggcgacagggtgactatcacctgccgcgcatcccaggatgtcaacaccgctgtggcatggtaccagcagaagcctggaaaagccccaaagctgctgatctacagcgcttccttcctgtattctggcgtgccaagtcggttttctggaagtagatcaggcactgacttcacactgactatctctagtctgcagcccgaagattttgccacctactattgccagcagcactataccacaccccctacattcggacagggcactaaagtggagattaagggcgggtcaggcggagggagcggaggagggtccggaggagggtctggaggagggagtggagaggtccagctggtggaatctggaggaggactggtgcagcctggaggctcactgcgactgagctgtgccgcttccggctttaacatcaaagacacatacattcattgggtcaggcaggcaccagggaagggactggaatgggtggcccgcatctatcccacaaatgggtacactcgatatgccgacagcgtgaaaggacggtttaccatttctgctgataccagtaagaacacagcatacctgcagatgaacagcctgcgcgcagaggatacagccgtgtactattgcagtcgatgggggggagacggcttctacgccatggattattggggccaggggactctggtcaccgtgtcaagcgcagccgaacctaaatcctctgacaagacccacacatgcccaccctgtcctgctccagagctgctgggaggaccatccgtgttcctgtttcctccaaagcctaaagatacactgatgattagccgcactcccgaagtcacctgtgtggtcgtggacgtgtcccacgaggaccccgaagtcaagttcaactggtacgtggacggcgtcgaggtgcataatgccaagactaaaccaagagaggaacagtacaattcaacctatagggtcgtgagcgtcctgacagtgctgcatcaggattggctgaacggcaaggagtataagtgcaaagtgtctaacaaggccctgcccgctcctatcgagaagactattagcaaggcaaaagggcagccacgggaaccccaggtctacgtgctgccccctagcagagacgagctgaccaaaaaccaggtctccctgctgtgtctggtgaagggcttttatcctagtgatatcgctgtggagtgggaatcaaatgggcagccagaaaacaattacctgacatggccacccgtgctggacagcgatgggtccttctttctgtattccaaactgactgtggacaagtctagatggcagcagggaaacgtcttcagctgttccgtgatgcacgaggccctgcacaatcattacacccagaagtctctgagtctgtcacccggc

SEQ ID NO: 65 - protein, 107 aa, Artificial Sequence [sequence omitted]

SEQ ID NO: 66 - protein, 120 aa, Artificial Sequence [sequence omitted]

SEQ ID NO: 67 - protein, 6 aa, Artificial Sequence
  Artificial sequence
QDVNTA

SEQ ID NO: 68 - protein, 3 aa, Artificial Sequence
  Artificial sequence
SAS

SEQ ID NO: 69 - protein, 9 aa, Artificial Sequence
  Artificial sequence
QQHYTTPPT

SEQ ID NO: 70 - protein, 8 aa, Artificial Sequence
  Artificial sequence
GFNIKDTY

SEQ ID NO: 71 - protein, 8 aa, Artificial Sequence
  Artificial sequence
IYPTNGYT

SEQ ID NO: 72 - protein, 13 aa, Artificial Sequence
  Artificial sequence
SRWGGDGFYAMDY

SEQ ID NO: 73 - protein, 8 aa, Artificial Sequence
  Artificial sequence
VNPNSGYS

SEQ ID NO: 74 - protein, 8 aa, Artificial Sequence
  Artificial sequence
GFTFQDYT

SEQ ID NO: 75 - protein, 12 aa, Artificial Sequence
  Artificial sequence
ARNLGPWFYFDY

SEQ ID NO: 76 - protein, 9 aa, Artificial Sequence
  Artificial sequence
QQYYIYPGT

SEQ ID NO: 77 - protein, 8 aa, Artificial Sequence
  Artificial sequence
GFTFYDYT

SEQ ID NO: 78 - protein, 119 aa, Artificial Sequence
  Artificial sequence
EVQLVESGGGLVQPGGSLRLSCAASGFTFADYTMDWVRQAPGKGLEWVADVNPNSGGSIYNQRFKGRFTLSVDRSKNTLYLQMNSLRAEDTAVYYCARNLGPSFYFDYWGQGTLVTVSS

SEQ ID NO: 79 - protein, 107 aa, Artificial Sequence; identical to SEQ ID NO: 26
  Artificial sequence

SEQ ID NO: 80 - protein, 119 aa, Artificial Sequence
  Artificial sequence
EVQLVESGGGLVQPGGSLRLSCAASGFTFTDYTMDWVRQAPGKGLEWVADVNPNSGYSIYNQRFKGRFTLSVDRSWNTLYLQMNSLRAEDTAVYYCARNLGPSFYFDYWGQGTLVTVSS

SEQ ID NO: 81 - protein, 107 aa, Artificial Sequence [sequence omitted]

SEQ ID NO: 82 - protein, 119 aa, Artificial Sequence
  Artificial sequence
EVQLVESGGGLVQPGGSLRLSCAASGFTFQDYTMDWVRQAPGKGLEWVADVNPNSGGSIYNQRFKGRFTLSVDRSKNTLYLQMNSLRAEDTAVYYCARNLGPWFYFDYWGQGTLVTVSS

SEQ ID NO: 83 - protein, 119 aa, Artificial Sequence
  Artificial sequence
EVQLVESGGGLVQPGGSLRLSCAASGFTFQDYTMDWVRQAPGKGLEWVADVNPNSGGSIYNQRFKGRFTLSVDRSKNTLYLQMNSLRAEDTAVYYCARNLGPSFYFDYWGQGTLVTVSS

SEQ ID NO: 84 - protein, 107 aa, Artificial Sequence
  Artificial sequence
DIQMTQSPSSLSASVGDRVTITCKASQDVSIGVAWYQQKPGKAPKLLIWSASYRYTGVPSRFSGSGSGTDFTLTISSLQPEDFATYYCQQYYIYPGTFGQGTKVEIK

SEQ ID NO: 85 - protein, 119 aa, Artificial Sequence
  Artificial sequence
EVQLVESGGGLVQPGGSLRLSCAASGFTFQDYTMDWVRQAPGKGLEWVADVNPNSGGSIYNQRFKGRFTLSVDRSWNTLYLQMNSLRAEDTAVYYCARNLGPSFYFDYWGQGTLVTVSS

SEQ ID NO: 86 - protein, 119 aa, Artificial Sequence
  Artificial sequence
EVQLVESGGGLVQPGGSLRLSCAASGFTFYDYTMDWVRQAPGKGLEWVADVNPNSGGSIYNQRFKGRFTLSVDRSWNTLYLQMNSLRAEDTAVYYCARNLGPSFYFDYWGQGTLVTVSS

SEQ ID NO: 87 - protein, 119 aa, Artificial Sequence
  Artificial sequence
EVQLVESGGGLVQPGGSLRLSCAASGFTFQDYTMDWVRQAPGKGLEWVADVNPNSGYSIYNQRFKGRFTLSVDRSKNTLYLQMNSLRAEDTAVYYCARNLGPWFYFDYWGQGTLVTVSS

SEQ ID NO: 88 - protein, 107 aa, Artificial Sequence
  Artificial sequence
DIQMTQSPSSLSASVGDRVTITCKASQDVSIGVAWYQQKPGKAPKLLIWSASYRYTGVPSRFSGSGSGTDFTLTISSLQPEDFATYYCQQYYIYPYTFGQGTKVEIK

SEQ ID NO: 89 - protein, 119 aa, Artificial Sequence
  Artificial sequence
EVQLVESGGGLVQPGGSLRLSCAASGFTFQDYTMDWVRQAPGKGLEWVADVNPNSGYSIYNQRFKGRFTLSVDRSKNTLYLQMNSLRAEDTAVYYCARNLGPSFYFDYWGQGTLVTVSS